European Patent Application EP 4 310 182 A1, published January 24, 2024. Title: PROTECTED DNA AND METHODS FOR THE PRODUCTION THEREOF. Applicant: 4basebio, S.L.U. The sequence listing filed with the application follows.

SEQUENCE LISTING (12 sequences)

SEQ ID NO: 1 - DNA, 17 bp, synthetic construct
  source 1..17: mol_type = other DNA
  modified_base 1: mod_base = OTHER; note = nuclease resistant nucleotide
nacaaatgttagccctn

SEQ ID NO: 2 - DNA, 17 bp, synthetic construct
  source 1..17: mol_type = other DNA
nagggctaacatttgtn

SEQ ID NO: 3 - DNA, 17 bp, synthetic construct
  source 1..17: mol_type = other DNA
  modified_base 17: mod_base = OTHER; note = nuclease resistant nucleotide
nagggctaacatttgtn

SEQ ID NO: 4 - DNA, 16 bp, synthetic construct
  source 1..16: mol_type = other DNA
  modified_base 16: mod_base = OTHER; note = nuclease resistant nucleotide
ncatgctaacatttgn

SEQ ID NO: 5 - DNA, 16 bp, synthetic construct
  source 1..16: mol_type = other DNA
ncaaatgttagcatgn

SEQ ID NO: 6 - DNA, 16 bp, synthetic construct
  source 1..16: mol_type = other DNA
  modified_base 1: mod_base = OTHER; note = nuclease resistant nucleotide
ncaaatgttagcatgn

SEQ ID NO: 7 - DNA, 12 bp, synthetic construct
  source 1..12: mol_type = other DNA
  modified_base 1: mod_base = OTHER; note = nuclease resistant nucleotide
nacaaatgttag

SEQ ID NO: 8 - DNA, 16 bp, synthetic construct
  source 1..16: mol_type = other DNA
agggctaacatttgtn

SEQ ID NO: 9 - DNA, 16 bp, synthetic construct
  source 1..16: mol_type = other DNA
  modified_base 16: mod_base = OTHER; note = nuclease resistant nucleotide
agggctaacatttgtn

SEQ ID NO: 10 - DNA, 15 bp, synthetic construct
  source 1..15: mol_type = other DNA
  modified_base 15: mod_base = OTHER; note = nuclease resistant nucleotide
catgctaacatttgn

SEQ ID NO: 11 - DNA, 11 bp, synthetic construct
  source 1..11: mol_type = other DNA
ncaaatgttag

SEQ ID NO: 12 - DNA, 11 bp, synthetic construct
  source 1..11: mol_type = other DNA
  modified_base 1: mod_base = OTHER; note = nuclease resistant nucleotide
ncaaatgttag